European Patent Application EP 4 623 995 A1, published October 1, 2025. Title: Monoclonal antibody, reagent for measuring Crtac1B, reagent kit, and method for measuring Crtac1B. Applicant: SYSMEX CORPORATION. Application JP 2024-045431, filed March 21, 2024. The sequence listing filed with the application follows.

SEQUENCE LISTING (30 sequences)

SEQ ID NO: 1 - protein, 8 aa, Mus musculus
GYTFTDYN

SEQ ID NO: 2 - protein, 8 aa, Mus musculus
INPNYDSS

SEQ ID NO: 3 - protein, 7 aa, Mus musculus
TRSGGTY

SEQ ID NO: 4 - protein, 6 aa, Mus musculus
QNINVW

SEQ ID NO: 5 - protein, 9 aa, Mus musculus
QQAQSYPRT

SEQ ID NO: 6 - protein, 114 aa, Mus musculus
EVQLQQFGAELVKPGASVKISCKASGYTFTDYNMDWVKQSHGKSLEWIGDINPNYDSSSYNQKFKGKATLTVDKSSSTAYMELRSLTSEDTAVYYCTRSGGTYWGQGTLVTVSA

SEQ ID NO: 7 - protein, 107 aa, Mus musculus
DIQMNQSPSSLSASLGDTITITCHASQNINVWLSWYQQKPGNIPKLLIYKASNLHTGVPSRFSGSGSGTGFSLTISSLQPEDIATYYCQQAQSYPRTFGGGTKLEIK

SEQ ID NO: 8 - protein, 645 aa, Homo sapiens
MAPSADPGMSRMLPFLLLLWFLPITEGSQRAEPMFTAVTNSVLPPDYDSNPTQLNYGVAVTDVDHDGDFEIVVAGYNGPNLVLKYDRAQKRLVNIAVDERSSPYYALRDRQGNAIGVTACDIDGDGREEIYFLNTNNAFSGVATYTDKLFKFRNNRWEDILSDEVNVARGVASLFAGRSVACVDRKGSGRYSIYIANYAYGNVGPDALIEMDPEASDLSRGILALRDVAAEAGVSKYTGGRGVSVGPILSSSASDIFCDNENGPNFLFHNRGDGTFVDAAASAGVDDPHQHGRGVALADFNRDGKVDIVYGNWNGPHRLYLQMSTHGKVRFRDIASPKFSMPSPVRTVITADFDNDQELEIFFNNIAYRSSSANRLFRVIRREHGDPLIEELNPGDALEPEGRGTGGVVTDFDGDGMLDLILSHGESMAQPLSVFRGNQGFNNNWLRVVPRTRFGAFARGAKVVLYTKKSGAHLRIIDGGSGYLCEMEPVAHFGLGKDEASSVEVTWPDGKMVSRNVASGEMNSVLEILYPRDEDTLQDPAPLECGQGFSQQENGHCMDTNECIQFPFVCPRDKPVCVNTYGSYRCRTNKKCSRGYEPNEDGTACVAQVAFLGGYSSAASRISEPLSRASYLSLGLGLCLQLYAL

SEQ ID NO: 9 - protein, 12 aa, Homo sapiens
ADGTACVAQVAA

SEQ ID NO: 10 - protein, 15 aa, synthetic construct
CPNEDGTAAVAQVAA

SEQ ID NO: 11 - protein, 20 aa, Homo sapiens
GCSRGYEPNEDGTACVAQVA

SEQ ID NO: 12 - protein, 614 aa, Homo sapiens
MAPSADPGMSRMLPFLLLLWFLPITEGSQRAEPMFTAVTNSVLPPDYDSNPTQLNYGVAVTDVDHDGDFEIVVAGYNGPNLVLKYDRAQKRLVNIAVDERSSPYYALRDRQGNAIGVTACDIDGDGREEIYFLNTNNAFSGVATYTDKLFKFRNNRWEDILSDEVNVARGVASLFAGRSVACVDRKGSGRYSIYIANYAYGNVGPDALIEMDPEASDLSRGILALRDVAAEAGVSKYTGGRGVSVGPILSSSASDIFCDNENGPNFLFHNRGDGTFVDAAASAGVDDPHQHGRGVALADFNRDGKVDIVYGNWNGPHRLYLQMSTHGKVRFRDIASPKFSMPSPVRTVITADFDNDQELEIFFNNIAYRSSSANRLFRVIRREHGDPLIEELNPGDALEPEGRGTGGVVTDFDGDGMLDLILSHGESMAQPLSVFRGNQGFNNNWLRVVPRTRFGAFARGAKVVLYTKKSGAHLRIIDGGSGYLCEMEPVAHFGLGKDEASSVEVTWPDGKMVSRNVASGEMNSVLEILYPRDEDTLQDPAPLECGQGFSQQENGHCMDTNECIQFPFVCPRDKPVCVNTYGSYRCRTNKKCSRGYEPNEDGTACVAQVAFLGG

SEQ ID NO: 13 - protein, 611 aa, Homo sapiens
MAPSADPGMSRMLPFLLLLWFLPITEGSQRAEPMFTAVTNSVLPPDYDSNPTQLNYGVAVTDVDHDGDFEIVVAGYNGPNLVLKYDRAQKRLVNIAVDERSSPYYALRDRQGNAIGVTACDIDGDGREEIYFLNTNNAFSGVATYTDKLFKFRNNRWEDILSDEVNVARGVASLFAGRSVACVDRKGSGRYSIYIANYAYGNVGPDALIEMDPEASDLSRGILALRDVAAEAGVSKYTGGRGVSVGPILSSSASDIFCDNENGPNFLFHNRGDGTFVDAAASAGVDDPHQHGRGVALADFNRDGKVDIVYGNWNGPHRLYLQMSTHGKVRFRDIASPKFSMPSPVRTVITADFDNDQELEIFFNNIAYRSSSANRLFRVIRREHGDPLIEELNPGDALEPEGRGTGGVVTDFDGDGMLDLILSHGESMAQPLSVFRGNQGFNNNWLRVVPRTRFGAFARGAKVVLYTKKSGAHLRIIDGGSGYLCEMEPVAHFGLGKDEASSVEVTWPDGKMVSRNVASGEMNSVLEILYPRDEDTLQDPAPLECGQGFSQQENGHCMDTNECIQFPFVCPRDKPVCVNTYGSYRCRTNKKCSRGYEPNEDGTACVAQVAF

SEQ ID NO: 14 - protein, 610 aa, Homo sapiens
MAPSADPGMSRMLPFLLLLWFLPITEGSQRAEPMFTAVTNSVLPPDYDSNPTQLNYGVAVTDVDHDGDFEIVVAGYNGPNLVLKYDRAQKRLVNIAVDERSSPYYALRDRQGNAIGVTACDIDGDGREEIYFLNTNNAFSGVATYTDKLFKFRNNRWEDILSDEVNVARGVASLFAGRSVACVDRKGSGRYSIYIANYAYGNVGPDALIEMDPEASDLSRGILALRDVAAEAGVSKYTGGRGVSVGPILSSSASDIFCDNENGPNFLFHNRGDGTFVDAAASAGVDDPHQHGRGVALADFNRDGKVDIVYGNWNGPHRLYLQMSTHGKVRFRDIASPKFSMPSPVRTVITADFDNDQELEIFFNNIAYRSSSANRLFRVIRREHGDPLIEELNPGDALEPEGRGTGGVVTDFDGDGMLDLILSHGESMAQPLSVFRGNQGFNNNWLRVVPRTRFGAFARGAKVVLYTKKSGAHLRIIDGGSGYLCEMEPVAHFGLGKDEASSVEVTWPDGKMVSRNVASGEMNSVLEILYPRDEDTLQDPAPLECGQGFSQQENGHCMDTNECIQFPFVCPRDKPVCVNTYGSYRCRTNKKCSRGYEPNEDGTACVAQVA

SEQ ID NO: 15 - protein, 609 aa, Homo sapiens
MAPSADPGMSRMLPFLLLLWFLPITEGSQRAEPMFTAVTNSVLPPDYDSNPTQLNYGVAVTDVDHDGDFEIVVAGYNGPNLVLKYDRAQKRLVNIAVDERSSPYYALRDRQGNAIGVTACDIDGDGREEIYFLNTNNAFSGVATYTDKLFKFRNNRWEDILSDEVNVARGVASLFAGRSVACVDRKGSGRYSIYIANYAYGNVGPDALIEMDPEASDLSRGILALRDVAAEAGVSKYTGGRGVSVGPILSSSASDIFCDNENGPNFLFHNRGDGTFVDAAASAGVDDPHQHGRGVALADFNRDGKVDIVYGNWNGPHRLYLQMSTHGKVRFRDIASPKFSMPSPVRTVITADFDNDQELEIFFNNIAYRSSSANRLFRVIRREHGDPLIEELNPGDALEPEGRGTGGVVTDFDGDGMLDLILSHGESMAQPLSVFRGNQGFNNNWLRVVPRTRFGAFARGAKVVLYTKKSGAHLRIIDGGSGYLCEMEPVAHFGLGKDEASSVEVTWPDGKMVSRNVASGEMNSVLEILYPRDEDTLQDPAPLECGQGFSQQENGHCMDTNECIQFPFVCPRDKPVCVNTYGSYRCRTNKKCSRGYEPNEDGTACVAQV

SEQ ID NO: 16 - protein, 608 aa, Homo sapiens
MAPSADPGMSRMLPFLLLLWFLPITEGSQRAEPMFTAVTNSVLPPDYDSNPTQLNYGVAVTDVDHDGDFEIVVAGYNGPNLVLKYDRAQKRLVNIAVDERSSPYYALRDRQGNAIGVTACDIDGDGREEIYFLNTNNAFSGVATYTDKLFKFRNNRWEDILSDEVNVARGVASLFAGRSVACVDRKGSGRYSIYIANYAYGNVGPDALIEMDPEASDLSRGILALRDVAAEAGVSKYTGGRGVSVGPILSSSASDIFCDNENGPNFLFHNRGDGTFVDAAASAGVDDPHQHGRGVALADFNRDGKVDIVYGNWNGPHRLYLQMSTHGKVRFRDIASPKFSMPSPVRTVITADFDNDQELEIFFNNIAYRSSSANRLFRVIRREHGDPLIEELNPGDALEPEGRGTGGVVTDFDGDGMLDLILSHGESMAQPLSVFRGNQGFNNNWLRVVPRTRFGAFARGAKVVLYTKKSGAHLRIIDGGSGYLCEMEPVAHFGLGKDEASSVEVTWPDGKMVSRNVASGEMNSVLEILYPRDEDTLQDPAPLECGQGFSQQENGHCMDTNECIQFPFVCPRDKPVCVNTYGSYRCRTNKKCSRGYEPNEDGTACVAQ

SEQ ID NO: 17 - protein, 607 aa, Homo sapiens
MAPSADPGMSRMLPFLLLLWFLPITEGSQRAEPMFTAVTNSVLPPDYDSNPTQLNYGVAVTDVDHDGDFEIVVAGYNGPNLVLKYDRAQKRLVNIAVDERSSPYYALRDRQGNAIGVTACDIDGDGREEIYFLNTNNAFSGVATYTDKLFKFRNNRWEDILSDEVNVARGVASLFAGRSVACVDRKGSGRYSIYIANYAYGNVGPDALIEMDPEASDLSRGILALRDVAAEAGVSKYTGGRGVSVGPILSSSASDIFCDNENGPNFLFHNRGDGTFVDAAASAGVDDPHQHGRGVALADFNRDGKVDIVYGNWNGPHRLYLQMSTHGKVRFRDIASPKFSMPSPVRTVITADFDNDQELEIFFNNIAYRSSSANRLFRVIRREHGDPLIEELNPGDALEPEGRGTGGVVTDFDGDGMLDLILSHGESMAQPLSVFRGNQGFNNNWLRVVPRTRFGAFARGAKVVLYTKKSGAHLRIIDGGSGYLCEMEPVAHFGLGKDEASSVEVTWPDGKMVSRNVASGEMNSVLEILYPRDEDTLQDPAPLECGQGFSQQENGHCMDTNECIQFPFVCPRDKPVCVNTYGSYRCRTNKKCSRGYEPNEDGTACVA

SEQ ID NO: 18 - protein, 606 aa, Homo sapiens
MAPSADPGMSRMLPFLLLLWFLPITEGSQRAEPMFTAVTNSVLPPDYDSNPTQLNYGVAVTDVDHDGDFEIVVAGYNGPNLVLKYDRAQKRLVNIAVDERSSPYYALRDRQGNAIGVTACDIDGDGREEIYFLNTNNAFSGVATYTDKLFKFRNNRWEDILSDEVNVARGVASLFAGRSVACVDRKGSGRYSIYIANYAYGNVGPDALIEMDPEASDLSRGILALRDVAAEAGVSKYTGGRGVSVGPILSSSASDIFCDNENGPNFLFHNRGDGTFVDAAASAGVDDPHQHGRGVALADFNRDGKVDIVYGNWNGPHRLYLQMSTHGKVRFRDIASPKFSMPSPVRTVITADFDNDQELEIFFNNIAYRSSSANRLFRVIRREHGDPLIEELNPGDALEPEGRGTGGVVTDFDGDGMLDLILSHGESMAQPLSVFRGNQGFNNNWLRVVPRTRFGAFARGAKVVLYTKKSGAHLRIIDGGSGYLCEMEPVAHFGLGKDEASSVEVTWPDGKMVSRNVASGEMNSVLEILYPRDEDTLQDPAPLECGQGFSQQENGHCMDTNECIQFPFVCPRDKPVCVNTYGSYRCRTNKKCSRGYEPNEDGTACV

SEQ ID NO: 19 - protein, 21 aa, Homo sapiens
RGYEPNEDGTACVAQVAFLGG

SEQ ID NO: 20 - protein, 18 aa, Homo sapiens
RGYEPNEDGTACVAQVAF

SEQ ID NO: 21 - protein, 17 aa, Homo sapiens
RGYEPNEDGTACVAQVA

SEQ ID NO: 22 - protein, 16 aa, Homo sapiens
RGYEPNEDGTACVAQV

SEQ ID NO: 23 - protein, 15 aa, Homo sapiens
RGYEPNEDGTACVAQ

SEQ ID NO: 24 - protein, 14 aa, Homo sapiens
RGYEPNEDGTACVA

SEQ ID NO: 25 - protein, 13 aa, Homo sapiens
RGYEPNEDGTACV

SEQ ID NO: 26 - DNA, 1371 bp, Mus musculus
  source 1..1371: mol_type = genomic DNA
atggaatggagctggatctttctctttctcctgtcaggaactgcaggtgtcctctctgaggtccagctgcaacagtttggagctgagctggtgaagcctggggcttcagtgaagatatcctgcaaggcttctggctacacattcactgactacaacatggactgggtgaagcagagccatggaaagagccttgagtggattggagatattaatcctaactatgatagttctagctacaaccagaagttcaagggaaaggccacattgactgtagacaagtcctccagcacagcctacatggagctccgcagcctgacatctgaggacactgcagtctattactgtacaagatcgggggggacttactggggccaagggactctggtcactgtctctgcagccaaaacgacacccccatctgtctatccactggcccctggatctgctgcccaaactaactccatggtgaccctgggatgcctggtcaagggctatttccctgagccagtgacagtgacctggaactctggatccctgtccagcggtgtgcacaccttcccagctgtcctgcagtctgacctctacactctgagcagctcagtgactgtcccctccagcacctggcccagcgagaccgtcacctgcaacgttgcccacccggccagcagcaccaaggtggacaagaaaattgtgcccagggattgtggttgtaagccttgcatatgtacagtcccagaagtatcatctgtcttcatcttccccccaaagcccaaggatgtgctcaccattactctgactcctaaggtcacgtgtgttgtggtagacatcagcaaggatgatcccgaggtccagttcagctggtttgtagatgatgtggaggtgcacacagctcagacgcaaccccgggaggagcagttcaacagcactttccgctcagtcagtgaacttcccatcatgcaccaggactggctcaatggcaaggagttcaaatgcagggtcaacagtgcagctttccctgcccccatcgagaaaaccatctccaaaaccaaaggcagaccgaaggctccacaggtgtacaccattccacctcccaaggagcagatggccaaggataaagtcagtctgacctgcatgataacagacttcttccctgaagacattactgtggagtggcagtggaatgggcagccagcggagaactacaagaacactcagcccatcatggacacagatggctcttacttcgtctacagcaagctcaatgtgcagaagagcaactgggaggcaggaaatactttcacctgctctgtgttacatgagggcctgcacaaccaccatactgagaagagcctctcccactctcctggtaaa

SEQ ID NO: 27 - DNA, 702 bp, Mus musculus
  source 1..702: mol_type = genomic DNA
atgagggtccttgctgagctcctggggctgctgctgttctgctttttaggtgtgagatgtgacatccagatgaaccagtctccatccagtctgtctgcatcccttggagacacaattaccatcacttgccatgccagtcagaacattaatgtttggttaagctggtaccagcagaaaccaggaaatattcctaaactattgatctataaggcttccaacttgcacacaggcgtcccatcaaggtttagtggcagtggatctggaacaggtttctcattaaccatcagcagcctgcagcctgaagacattgccacttactactgtcaacaggctcaaagttatcctcggacgttcggtggaggcaccaagctggaaatcaagcgggctgatgctgcaccaactgtatccatcttcccaccatccagtgagcagttaacatctggaggtgcctcagtcgtgtgcttcttgaacaacttctaccccaaagacatcaatgtcaagtggaagattgatggcagtgaacgacaaaatggcgtcctgaacagttggactgatcaggacagcaaagacagcacctacagcatgagcagcaccctcacgttgaccaaggacgagtatgaacgacataacagctatacctgtgaggccactcacaagacatcaacttcacccattgtcaagagcttcaacaggaatgagtgt

SEQ ID NO: 28 - protein, 457 aa, Mus musculus
MEWSWIFLFLLSGTAGVLSEVQLQQFGAELVKPGASVKISCKASGYTFTDYNMDWVKQSHGKSLEWIGDINPNYDSSSYNQKFKGKATLTVDKSSSTAYMELRSLTSEDTAVYYCTRSGGTYWGQGTLVTVSAAKTTPPSVYPLAPGSAAQTNSMVTLGCLVKGYFPEPVTVTWNSGSLSSGVHTFPAVLQSDLYTLSSSVTVPSSTWPSETVTCNVAHPASSTKVDKKIVPRDCGCKPCICTVPEVSSVFIFPPKPKDVLTITLTPKVTCVVVDISKDDPEVQFSWFVDDVEVHTAQTQPREEQFNSTFRSVSELPIMHQDWLNGKEFKCRVNSAAFPAPIEKTISKTKGRPKAPQVYTIPPPKEQMAKDKVSLTCMITDFFPEDITVEWQWNGQPAENYKNTQPIMDTDGSYFVYSKLNVQKSNWEAGNTFTCSVLHEGLHNHHTEKSLSHSPGK

SEQ ID NO: 29 - protein, 234 aa, Mus musculus
MRVLAELLGLLLFCFLGVRCDIQMNQSPSSLSASLGDTITITCHASQNINVWLSWYQQKPGNIPKLLIYKASNLHTGVPSRFSGSGSGTGFSLTISSLQPEDIATYYCQQAQSYPRTFGGGTKLEIKRADAAPTVSIFPPSSEQLTSGGASVVCFLNNFYPKDINVKWKIDGSERQNGVLNSWTDQDSKDSTYSMSSTLTLTKDEYERHNSYTCEATHKTSTSPIVKSFNRNEC

SEQ ID NO: 30 - protein, 661 aa, Homo sapiens
MAPSADPGMSRMLPFLLLLWFLPITEGSQRAEPMFTAVTNSVLPPDYDSNPTQLNYGVAVTDVDHDGDFEIVVAGYNGPNLVLKYDRAQKRLVNIAVDERSSPYYALRDRQGNAIGVTACDIDGDGREEIYFLNTNNAFSGVATYTDKLFKFRNNRWEDILSDEVNVARGVASLFAGRSVACVDRKGSGRYSIYIANYAYGNVGPDALIEMDPEASDLSRGILALRDVAAEAGVSKYTGGRGVSVGPILSSSASDIFCDNENGPNFLFHNRGDGTFVDAAASAGVDDPHQHGRGVALADFNRDGKVDIVYGNWNGPHRLYLQMSTHGKVRFRDIASPKFSMPSPVRTVITADFDNDQELEIFFNNIAYRSSSANRLFRVIRREHGDPLIEELNPGDALEPEGRGTGGVVTDFDGDGMLDLILSHGESMAQPLSVFRGNQGFNNNWLRVVPRTRFGAFARGAKVVLYTKKSGAHLRIIDGGSGYLCEMEPVAHFGLGKDEASSVEVTWPDGKMVSRNVASGEMNSVLEILYPRDEDTLQDPAPLECGQGFSQQENGHCMDTNECIQFPFVCPRDKPVCVNTYGSYRCRTNKKCSRGYEPNEDGTACVGTLGQSPGPRPTTPTAAAATAAAAAAAGAATAAPVLVDGDLNLGSVVKESCEPSC